European Patent Specification EP 3 897 697 B1, published March 29, 2023. Title: PEPTIDES FOR TREATMENT AND PREVENTION OF DIABETES AND ASSOCIATED DISORDERS. Applicant: Université de Strasbourg et al. The sequence listing filed with the application follows.

SEQUENCE LISTING (57 sequences)

SEQ ID NO: 1 - protein, 672 aa, Homo sapiens
MADVFPGNDSTASQDVANRFARKGALRQKNVHEVKDHKFIARFFKQPTFCSHCTDFIWGFGKQGFQCQVCCFVVHKRCHEFVTFSCPGADKGPDTDDPRSKHKFKIHTYGSPTFCDHCGSLLYGLIHQGMKCDTCDMNVHKQCVINVPSLCGMDHTEKRGRIYLKAEVADEKLHVTVRDAKNLIPMDPNGLSDPYVKLKLIPDPKNESKQKTKTIRSTLNPQWNESFTFKLKPSDKDRRLSVEIWDWDRTTRNDFMGSLSFGVSELMKMPASGWYKLLNQEEGEYYNVPIPEGDEEGNMELRQKFEKAKLGPAGNKVISPSEDRKQPSNNLDRVKLTDFNFLMVLGKGSFGKVMLADRKGTEELYAIKILKKDVVIQDDDVECTMVEKRVLALLDKPPFLTQLHSCFQTVDRLYFVMEYVNGGDLMYHIQQVGKFKEPQAVFYAAEISIGLFFLHKRGIIYRDLKLDNVMLDSEGHIKIADFGMCKEHMMDGVTTRTFCGTPDYIAPEIIAYQPYGKSVDWWAYGVLLYEMLAGQPPFDGEDEDELFQSIMEHNVSYPKSLSKEAVSVCKGLMTKHPAKRLGCGPEGERDVREHAFFRRIDWEKLENREIQPPFKPKVCGKGAENFDKFFTRGQPVLTPPDQLVIANIDQSDFEGFSYVNPQFVHPILQSAV

SEQ ID NO: 2 - protein, 257 aa, Homo sapiens
FNFLMVLGKGSFGKVMLADRKGTEELYAIKILKKDVVIQDDDVECTMVEKRVLALLDKPPFLTQLHSCFQTVDRLYFVMEYVNGGDLMYHIQQVGKFKEPQAVFYAAEISIGLFFLHKRGIIYRDLKLDNVMLDSEGHIKIADFGMCKEHMMDGVTTRTFCGTPDYIAPEIIAYQPYGKSVDWWAYGVLLYEMLAGQPPFDGEDEDELFQSIMEHNVSYPKSLSKEAVSVCKGLMTKHPAKRLGCGPEGERDVREHA

SEQ ID NO: 3 - protein, 12 aa, artificial sequence
  segment of kinase domain of alphaPKC
VECTMVEKRVLA

SEQ ID NO: 4 - protein, 8 aa, artificial sequence
  segment of kinase domain of alphaPKC
LMYHIQQV

SEQ ID NO: 5 - protein, 4 aa, artificial sequence
  segment of kinase domain of alphaPKC
PEII

SEQ ID NO: 6 - protein, 16 aa, artificial sequence
  segment of kinase domain of alphaPKC
SVDWWAYGVLLYEMLA

SEQ ID NO: 7 - protein, 12 aa, artificial sequence
  segment of kinase domain of alphaPKC
EDEDELFQSIME

SEQ ID NO: 8 - protein, 7 aa, artificial sequence
  segment of kinase domain of alphaPKC
GERDVRE

SEQ ID NO: 9 - protein, 12 aa, artificial sequence
  mutated segment of kinase domain of alphaPKC
  MISC_FEATURE (5)..(5): Xaa is any amino acid except R, M and P
VECTXVEKRVLA

SEQ ID NO: 10 - protein, 12 aa, artificial sequence
  mutated segment of kinase domain of alphaPKC
  MISC_FEATURE (9)..(9): Xaa is any amino acid except M, P and R
VECTMVEKXVLA

SEQ ID NO: 11 - protein, 12 aa, artificial sequence
  mutated segment of kinase domain of alphaPKC
  MISC_FEATURE (5)..(5): Xaa is any amino acid except M, P and R
  MISC_FEATURE (9)..(9): Xaa is any amino acid except M, P and R
VECTXVEKXVLA

SEQ ID NO: 12 - protein, 8 aa, artificial sequence
  mutated segment of kinase domain of alphaPKC
  MISC_FEATURE (2)..(2): Xaa is any amino acid except M, P and R
LXYHIQQV

SEQ ID NO: 13 - protein, 16 aa, artificial sequence
  mutated segment of kinase domain of alphaPKC
  MISC_FEATURE (14)..(14): Xaa is any amino acid except M, P and R
SVDWWAYGVLLYEXLA

SEQ ID NO: 14 - protein, 12 aa, artificial sequence
  mutated segment of kinase domain of alphaPKC
  MISC_FEATURE (11)..(11): Xaa is any amino acid except M, P and R
EDEDELFQSIXE

SEQ ID NO: 15 - protein, 7 aa, artificial sequence
  mutated segment of kinase domain of alphaPKC
  MISC_FEATURE (3)..(3): Xaa is any amino acid except M, P and R
GEXDVRE

SEQ ID NO: 16 - protein, 7 aa, artificial sequence
  mutated segment of kinase domain of alphaPKC
  MISC_FEATURE (6)..(6): Xaa is any amino acid except M, P and R
GERDVXE

SEQ ID NO: 17 - protein, 7 aa, artificial sequence
  mutated segment of kinase domain of alphaPKC
  MISC_FEATURE (3)..(3): Xaa is any amino acid except M, P and R
  MISC_FEATURE (6)..(6): Xaa is any amino acid except M, P and R
GEXDVXE

SEQ ID NO: 18 - protein, 4 aa, artificial sequence
  mutated segment of kinase domain of alphaPKC
  MISC_FEATURE (1)..(1): Xaa is any amino acid except M, P and R
XEII

SEQ ID NO: 19 - protein, 12 aa, artificial sequence
  mutated segment of kinase domain of alphaPKC
VECTTVEKEVLA

SEQ ID NO: 20 - protein, 25 aa, artificial sequence
  mutated segment of kinase domain of alphaPKC
  MISC_FEATURE (5)..(5): Xaa is any amino acid except M, P and R
  MISC_FEATURE (9)..(9): Xaa is any amino acid except M, P and R
  MISC_FEATURE (17)..(18): Xaa is any amino acid except M, P and R
VECTXVEKXVLALLDKXXFLTQLHS

SEQ ID NO: 21 - protein, 25 aa, artificial sequence
  mutated segment of kinase domain of alphaPKC
  MISC_FEATURE (17)..(18): Xaa is any amino acid except M, P and R
VECTMVEKRVLALLDKXXFLTQLHS

SEQ ID NO: 22 - protein, 25 aa, artificial sequence
  mutated segment of kinase domain of alphaPKC
  MISC_FEATURE (5)..(5): Xaa is any amino acid except M, P and R
VECTXVEKRVLALLDKPPFLTQLHS

SEQ ID NO: 23 - protein, 25 aa, artificial sequence
  mutated segment of kinase domain of alphaPKC
  MISC_FEATURE (9)..(9): Xaa is any amino acid except M, P and R
VECTMVEKXVLALLDKPPFLTQLHS

SEQ ID NO: 24 - protein, 13 aa, artificial sequence
  mutated segment of kinase domain of alphaPKC
  MISC_FEATURE (6)..(6): Xaa is any amino acid derivative suitable for stapling
  MISC_FEATURE (13)..(13): Xaa is any amino acid derivative suitable for stapling
VECTMXEKRVLAX

SEQ ID NO: 25 - protein, 13 aa, artificial sequence
  mutated segment of kinase domain of alphaPKC
  MISC_FEATURE (5)..(5): Xaa is any amino acid except M, P and R
  MISC_FEATURE (6)..(6): Xaa is any amino acid derivative suitable for stapling
  MISC_FEATURE (13)..(13): Xaa is any amino acid derivative suitable for stapling
VECTXXEKRVLAX

SEQ ID NO: 26 - protein, 13 aa, artificial sequence
  mutated segment of kinase domain of alphaPKC
  MISC_FEATURE (6)..(6): Xaa is any amino acid derivative suitable for stapling
  MISC_FEATURE (9)..(9): Xaa is any amino acid except M, P and R
  MISC_FEATURE (13)..(13): Xaa is any amino acid derivative suitable for stapling
VECTMXEKXVLAX

SEQ ID NO: 27 - protein, 13 aa, artificial sequence
  mutated segment of kinase domain of alphaPKC
  MISC_FEATURE (5)..(5): Xaa is any amino acid except M, P and R
  MISC_FEATURE (6)..(6): Xaa is any amino acid derivative suitable for stapling
  MISC_FEATURE (9)..(9): Xaa is any amino acid except M, P and R
  MISC_FEATURE (13)..(13): Xaa is any amino acid derivative suitable for stapling
VECTXXEKXVLAX

SEQ ID NO: 28 - protein, 25 aa, artificial sequence
  mutated segment of kinase domain of alphaPKC
  MISC_FEATURE (5)..(5): Xaa is any amino acid except M, P and R
  MISC_FEATURE (6)..(6): Xaa is any amino acid derivative suitable for stapling
  MISC_FEATURE (9)..(9): Xaa is any amino acid except M, P and R
  MISC_FEATURE (13)..(13): Xaa is any amino acid derivative suitable for stapling
  MISC_FEATURE (17)..(18): Xaa is any amino acid except M, P and R
VECTXXEKXVLAXLDKXXFLTQLHS

SEQ ID NO: 29 - protein, 25 aa, artificial sequence
  mutated segment of kinase domain of alphaPKC
  MISC_FEATURE (6)..(6): Xaa is any amino acid derivative suitable for stapling
  MISC_FEATURE (13)..(13): Xaa is any amino acid derivative suitable for stapling
  MISC_FEATURE (17)..(18): Xaa is any amino acid except M, P and R
VECTMXEKRVLAXLDKXXFLTQLHS

SEQ ID NO: 30 - protein, 25 aa, artificial sequence
  mutated segment of kinase domain of alphaPKC
  MISC_FEATURE (5)..(5): Xaa is any amino acid except M, P and R
  MISC_FEATURE (6)..(6): Xaa is any amino acid derivative suitable for stapling
  MISC_FEATURE (13)..(13): Xaa is any amino acid derivative suitable for stapling
VECTXXEKRVLAXLDKPPFLTQLHS

SEQ ID NO: 31 - protein, 25 aa, artificial sequence
  mutated segment of kinase domain of alphaPKC
  MISC_FEATURE (6)..(6): Xaa is any amino acid derivative suitable for stapling
  MISC_FEATURE (9)..(9): Xaa is any amino acid except M, P and R
  MISC_FEATURE (13)..(13): Xaa is any amino acid derivative suitable for stapling
VECTMXEKXVLAXLDKPPFLTQLHS

SEQ ID NO: 32 - protein, 25 aa, artificial sequence
  mutated segment of kinase domain of alphaPKC
VECTTREKEVLASLDKAAFLTQLHS

SEQ ID NO: 33 - protein, 8 aa, artificial sequence
  protein transduction domain
RRRRRRRR

SEQ ID NO: 34 - protein, 15 aa, artificial sequence
  protein transduction domain
RRPRRPRRPRRPRRP

SEQ ID NO: 35 - protein, 16 aa, artificial sequence
  penetratin peptide
RQIKIWFQNRRMKWKK

SEQ ID NO: 36 - protein, 11 aa, artificial sequence
  HIV-tat
YGRKKRRQRRR

SEQ ID NO: 37 - DNA, 20 bp, artificial sequence
  primer
tgctttggtttctgggactt

SEQ ID NO: 38 - DNA, 20 bp, artificial sequence
  primer
gctctagccgaacacgaatc

SEQ ID NO: 39 - DNA, 22 bp, artificial sequence
  primer
tggacaaagtagacggagtgtc

SEQ ID NO: 40 - DNA, 20 bp, artificial sequence
  primer
tagcaaggcctgtcccatac

SEQ ID NO: 41 - DNA, 20 bp, artificial sequence
  primer
tgagaacttgccaccgtatg

SEQ ID NO: 42 - DNA, 20 bp, artificial sequence
  primer
ggcaggtaggcccctatatc

SEQ ID NO: 43 - DNA, 20 bp, artificial sequence
  primer
gtttcatccgggtcttcatc

SEQ ID NO: 44 - DNA, 20 bp, artificial sequence
  primer
gtgtctgtgccctcgaaaat

SEQ ID NO: 45 - DNA, 20 bp, artificial sequence
  primer
aagttctctgcctcccgatt

SEQ ID NO: 46 - DNA, 20 bp, artificial sequence
  primer
caaagcgttgctggaagttt

SEQ ID NO: 47 - DNA, 20 bp, artificial sequence
  primer
tcgattccctcctacactgc

SEQ ID NO: 48 - DNA, 20 bp, artificial sequence
  primer
ttggtggtactggctcatca

SEQ ID NO: 49 - protein, 25 aa, artificial sequence
  PATAD
VECTMAEKRVLAALDKPPFLTQLHS

SEQ ID NO: 50 - protein, 13 aa, artificial
  segment of kinase domain of alphaPKC
ECTMVEKKVLALL

SEQ ID NO: 51 - protein, 15 aa, artificial
  mutated segment of kinase domain of alphaPKC
SVEWWAYGLLYEMLA

SEQ ID NO: 52 - protein, 15 aa, artificial
  mutated segment of kinase domain of alphaPKC
  MISC_FEATURE (3)..(3): Xaa is any amino acid except M, P and R
SVXWWAYGLLYEMLA

SEQ ID NO: 53 - protein, 24 aa, artificial
  mutated segment of kinase domain of alphaPKC
  MISC_FEATURE (6)..(6): Xaa is any amino acid derivative suitable for stapling
  MISC_FEATURE (13)..(13): Xaa is any amino acid derivative suitable for stapling
VECTTXEKEVLAXLDKAAFLTQHS

SEQ ID NO: 54 - protein, 19 aa, artificial
  mutated segment of kinase domain of alphaPKC
  MISC_FEATURE (6)..(6): Xaa is any amino acid derivative suitable for stapling
  MISC_FEATURE (13)..(13): Xaa is any amino acid derivative suitable for stapling
VECTTXEKEVLAXLDKAAF

SEQ ID NO: 55 - protein, 19 aa, artificial
  mutated segment of kinase domain of alphaPKC
  MISC_FEATURE (6)..(6): Xaa is any amino acid derivative suitable for stapling
  MISC_FEATURE (13)..(13): Xaa is any amino acid derivative suitable for stapling
VEGTTXEKEVLAXLDKAAF

SEQ ID NO: 56 - protein, 13 aa, artificial
  mutated segment of kinase domain of alphaPKC
  MISC_FEATURE (4)..(4): Xaa is any amino acid derivative suitable for stapling
  misc_feature (5)..(5): Xaa can be any naturally occurring amino acid
  MISC_FEATURE (12)..(12): Xaa is any amino acid derivative suitable for stapling
ECTTXEKEVLAXL

SEQ ID NO: 57 - protein, 13 aa, artificial
  mutated segment of kinase domain of alphaPKC
  MISC_FEATURE (4)..(4): Xaa is any amino acid derivative suitable for stapling
  misc_feature (5)..(5): Xaa can be any naturally occurring amino acid
  MISC_FEATURE (12)..(12): Xaa is any amino acid derivative suitable for stapling
ECTMXEKKVLAXL